European Patent Specification EP 3 408 412 B1, published March 20, 2024. Title: METHODS FOR ASSESSING RISK OF DEVELOPING COLORECTAL CANCER. Applicant: The University of Melbourne. The sequence listing filed with the application follows.

SEQUENCE LISTING (12 sequences)

SEQ ID NO: 1 - DNA, 19 bp, Artificial Sequence
  Artificial Sequence
tgcagcaagtggtgagaag

SEQ ID NO: 2 - DNA, 24 bp, Artificial Sequence
  Artificial Sequence
cccattgttaccagtatgaagagt

SEQ ID NO: 3 - DNA, 22 bp, Artificial Sequence
  Artificial Sequence
agacactctcctctgttgattt

SEQ ID NO: 4 - DNA, 24 bp, Artificial Sequence
  Artificial Sequence
ggacatcaaataatgtgcctagaa

SEQ ID NO: 5 - DNA, 20 bp, Artificial Sequence
  Artificial Sequence
cctgagtagctgggactaca

SEQ ID NO: 6 - DNA, 19 bp, Artificial Sequence
  Artificial Sequence
tcgagaccatcctggctaa

SEQ ID NO: 7 - DNA, 18 bp, Artificial Sequence
  Artificial Sequence
aacggtcagacgcaaaca

SEQ ID NO: 8 - DNA, 23 bp, Artificial Sequence
  Artificial Sequence
gacggcaataaatcttccatgag

SEQ ID NO: 9 - DNA, 21 bp, Artificial Sequence
  Artificial Sequence
cctttgagctcagcagatgaa

SEQ ID NO: 10 - DNA, 19 bp, Artificial Sequence
  Artificial Sequence
gggttcctgccctttgatt

SEQ ID NO: 11 - DNA, 20 bp, Artificial Sequence
  Artificial Sequence
ttgggccacacagtctctaa

SEQ ID NO: 12 - DNA, 21 bp, Artificial Sequence
  Artificial Sequence
tgagttgctgtggctgtaatg